European Patent Specification EP 3 873 524 B1, published February 26, 2025. Title: METHODS OF TREATMENT USING ANTI-CD123 IMMUNOCONJUGATES. Applicant: ImmunoGen, Inc. The sequence listing filed with the application follows.

SEQUENCE LISTING (12 sequences)

SEQ ID NO: 1 - protein, 121 aa, Artificial Sequence
  huCD123-6Gv7 Heavy Chain Variable Region
QVQLVQSGAEVKKPGASVKVSCKASGYIFTSSIMHWVRQAPGQGLEWIGYIKPYNDGTKYNEKFKGRATLTSDRSTSTAYMELSSLRSEDTAVYYCAREGGNDYYDTMDYWGQGTLVTVSS

SEQ ID NO: 2 - protein, 108 aa, Artificial Sequence
  huCD123-6Gv4 Light Chain Variable Region
DIQMTQSPSSLSASVGDRVTITCRASQDINSYLSWFQQKPGKAPKTLIYRVNRLVDGVPSRFSGSGSGNDYTLTISSLQPEDFATYYCLQYDAFPYTFGQGTKVEIKR

SEQ ID NO: 3 - protein, 450 aa, Artificial Sequence
  huCD123-6Gv7-C442 Full Length Heavy Chain
QVQLVQSGAEVKKPGASVKVSCKASGYIFTSSIMHWVRQAPGQGLEWIGYIKPYNDGTKYNEKFKGRATLTSDRSTSTAYMELSSLRSEDTAVYYCAREGGNDYYDTMDYWGQGTLVTVSSASTKGPSVFPLAPSSKSTSGGTAALGCLVKDYFPEPVTVSWNSGALTSGVHTFPAVLQSSGLYSLSSVVTVPSSSLGTQTYICNVNHKPSNTKVDKKVEPKSCDKTHTCPPCPAPELLGGPSVFLFPPKPKDTLMISRTPEVTCVVVDVSHEDPEVKFNWYVDGVEVHNAKTKPREEQYNSTYRVVSVLTVLHQDWLNGKEYKCKVSNKALPAPIEKTISKAKGQPREPQVYTLPPSRDELTKNQVSLTCLVKGFYPSDIAVEWESNGQPENNYKTTPPVLDSDGSFFLYSKLTVDKSRWQQGNVFSCSVMHEALHNHYTQKSLCLSPG

SEQ ID NO: 4 - protein, 214 aa, Artificial Sequence
  huCD123-6Gv4 Full Length Light Chain
DIQMTQSPSSLSASVGDRVTITCRASQDINSYLSWFQQKPGKAPKTLIYRVNRLVDGVPSRFSGSGSGNDYTLTISSLQPEDFATYYCLQYDAFPYTFGQGTKVEIKRTVAAPSVFIFPPSDEQLKSGTASVVCLLNNFYPREAKVQWKVDNALQSGNSQESVTEQDSKDSTYSLSSTLTLSKADYEKHKVYACEVTHQGLSSPVTKSFNRGEC

SEQ ID NO: 5 - protein, 5 aa, Artificial Sequence
  huCD123-6Gv7 Variable Heavy Chain CDR1
SSIMH

SEQ ID NO: 6 - protein, 17 aa, Artificial Sequence
  huCD123-6Gv7 Variable Heavy Chain CDR2
YIKPYNDGTKYNEKFKG

SEQ ID NO: 7 - protein, 12 aa, Artificial Sequence
  huCD123-6Gv7 Variable Heavy Chain CDR3
EGGNDYYDTMDY

SEQ ID NO: 8 - protein, 11 aa, Artificial Sequence
  huCD123-6Gv4 Variable Light Chain CDR1
RASQDINSYLS

SEQ ID NO: 9 - protein, 7 aa, Artificial Sequence
  huCD123-6Gv4 Variable Light Chain CDR2
RVNRLVD

SEQ ID NO: 10 - protein, 9 aa, Artificial Sequence
  huCD123-6Gv4 Variable Light Chain CDR3
LQYDAFPYT

SEQ ID NO: 11 - protein, 378 aa, Homo sapiens
MVLLWLTLLLIALPCLLQTKEDPNPPITNLRMKAKAQQLTWDLNRNVTDIECVKDADYSMPAVNNSYCQFGAISLCEVTNYTVRVANPPFSTWILFPENSGKPWAGAENLTCWIHDVDFLSCSWAVGPGAPADVQYDLYLNVANRRQQYECLHYKTDAQGTRIGCRFDDISRLSSGSQSSHILVRGRSAAFGIPCTDKFVVFSQIEILTPPNMTAKCNKTHSFMHWKMRSHFNRKFRYELQIQKRMQPVITEQVRDRTSFQLLNPGTYTVQIRARERVYEFLSAWSTPQRFECDQEEGANTRAWRTSLLIALGTLLALVCVFVICRRYLVMQRLFPRIPHMKDPIGDSFQNDKLVVWEAGKAGLEECLVTEVQVVQKT

SEQ ID NO: 12 - protein, 300 aa, Homo sapiens
MVLLWLTLLLIALPCLLQTKEGGKPWAGAENLTCWIHDVDFLSCSWAVGPGAPADVQYDLYLNVANRRQQYECLHYKTDAQGTRIGCRFDDISRLSSGSQSSHILVRGRSAAFGIPCTDKFVVFSQIEILTPPNMTAKCNKTHSFMHWKMRSHFNRKFRYELQIQKRMQPVITEQVRDRTSFQLLNPGTYTVQIRARERVYEFLSAWSTPQRFECDQEEGANTRAWRTSLLIALGTLLALVCVFVICRRYLVMQRLFPRIPHMKDPIGDSFQNDKLVVWEAGKAGLEECLVTEVQVVQKT